European Patent Specification EP 3 303 598 B1, published March 19, 2025. Title: TARGETED LIPID PARTICLES FOR SYSTEMIC DELIVERY OF NUCLEIC ACID MOLECULES TO LEUKOCYTES. Applicant: RAMOT at Tel-Aviv University Ltd. The sequence listing filed with the application follows.

SEQUENCE LISTING (19 sequences)

SEQ ID NO: 1 - DNA, 24 bp, Artificial Sequence
  Chemically modified siRNAs sequences
cuggcugaauuucagagcadtsdt

SEQ ID NO: 2 - DNA, 24 bp, Artificial Sequence
  Chemically modified siRNAs sequence
ugcucugaaauucagccagdtsdt

SEQ ID NO: 3 - DNA, 24 bp, Artificial Sequence
  Chemically modified siRNAs sequence
cuuacgcugaguacuucgadtsdt

SEQ ID NO: 4 - DNA, 24 bp, Artificial Sequence
  Chemically modified siRNAs sequence
ucgaaguacucagcguaagdtsdt

SEQ ID NO: 5 - DNA, 21 bp, Artificial Sequence
  Chemically modified siRNAs sequence
guaggacucucauucgggatt

SEQ ID NO: 6 - DNA, 22 bp, Artificial Sequence
  Primer
ccatcgtgtcatcaaggacttc

SEQ ID NO: 7 - DNA, 21 bp, Artificial Sequence
  Primer
gatgctctttcctcctgtgcc

SEQ ID NO: 8 - DNA, 22 bp, Artificial Sequence
  Primer
tcttacaccatccactctgggc

SEQ ID NO: 9 - DNA, 23 bp, Artificial Sequence
  Primer
gcttcgttgtggtagctatggtt

SEQ ID NO: 10 - DNA, 20 bp, Artificial Sequence
  Primer
gaggagccccaacaacttcc

SEQ ID NO: 11 - DNA, 21 bp, Artificial Sequence
  Primer
gtccgggtcacacttgatcac

SEQ ID NO: 12 - DNA, 20 bp, Artificial Sequence
  Primer
cgcaagcatgctcagacctt

SEQ ID NO: 13 - DNA, 18 bp, Artificial Sequence
  Primer
tgcgatcatcgacggtgg

SEQ ID NO: 14 - DNA, 23 bp, Artificial Sequence
  Primer
ctgaccatcgaaaaactgtgcat

SEQ ID NO: 15 - DNA, 17 bp, Artificial Sequence
  Primer
acctcccagtcccgcaa

SEQ ID NO: 16 - DNA, 20 bp, Artificial Sequence
  Primer
tccagagagccagtccatgc

SEQ ID NO: 17 - DNA, 19 bp, Artificial Sequence
  Primer
cctgccacaattccatgct

SEQ ID NO: 18 - DNA, 22 bp, Artificial Sequence
  Primer
accaagagagttgtccgcagtg

SEQ ID NO: 19 - DNA, 21 bp, Artificial Sequence
  Primer
tcatggcattacggatggtcc